European Patent Specification EP 4 171 199 B1, published January 28, 2026. Title: SWEET PROTEIN FROM TRUFFLE. Applicant: MycoTechnology, Inc. The sequence listing filed with the application follows.

SEQUENCE LISTING (75 sequences)

SEQ ID NO: 1 - DNA, 1072 bp, Mattirolomyces terfezioides
caagtctttaagtgttgatcgagcagtagaaatattaatcgcccaattaattgctcttactctaggaaatgtagtactcaagttggccctctaagtccctgattcagtgtcactttttctcctttgacagtaggctagattctagctcttgtgtccgtttcttaaaatcctgatatggcaccttagcgtcagagcagaatacctgttctcatacaccttggctatgatccgatatttaaatagagcaatcacccttctggatatcttccccatagctcccattgacctcaaacattttctaatcccctataccagccatattacttgtctaagcacttcacattcttcctcacaatacgaaacctcctaaaatgcctgatctctcctccttcattacgattaagaacaactctaaccacgtcttcactcggacggcaatttattctaagtatgccgctgtgcagtggagtcccgagccgcaactctcaatctctcccggcaaatgggatttgtttattttaaaggacatcttgtctatccgtgggacttcgggatatgtacaatatcgggttggggatggtcctggatgggttagggtcaccttttcttctctagtcggggccgatgaagtggcagagtggagctcaggtgacctacctgatggctttgttctccaaaaaccagttcgcactgggtccaggcctttgcaggcaacgttcgaggctacaaaacagtaaagatcgatgatgcctaatatgcctccataacactgacccgcgtgcacatggccgcatgaatgataagggggatatcgatgatgatgggattagttattggaattttcacaatggacgtcggcttggatttacaataatcgtttcatttgtattcaaatattcctatttccttgggtttttgtatttatctccttcatcacgccttctgaggccgtgggaagatgaatatgtaatcaaaagaagttaggatatgcatcatgtacagaaagtggaccgcaaccccttcagcgaaatgttataaagatgatatctaagacgccaaagcacattctcag

SEQ ID NO: 2 - DNA, 366 bp, Mattirolomyces terfezioides
atgcctgatctctcctccttcattacgattaagaacaactctaaccacgtcttcactcggacggcaatttattctaagtatgccgctgtgcagtggagtcccgagccgcaactctcaatctctcccggcaaatgggatttgtttattttaaaggacatcttgtctatccgtgggacttcgggatatgtacaatatcgggttggggatggtcctggatgggttagggtcaccttttcttctctagtcggggccgatgaagtggcagagtggagctcaggtgacctacctgatggctttgttctccaaaaaccagttcgcactgggtccaggcctttgcaggcaacgttcgaggctacaaaacagtaa

SEQ ID NO: 3 - protein, 121 aa, Mattirolomyces terfezioides [sequence omitted]

SEQ ID NO: 4 - protein, 20 aa, Mattirolomyces terfezioides
PDLSSFITIKNNSNHVFTRT

SEQ ID NO: 5 - DNA, 873 bp, Pisolithus tincturius
tcgtccgagcagataaacatcgacgggcaggatgtcatttctactgaatgtctggaacgctgtccaggcccgaggtacaatcttcctatcaacgacgcagacgaggtacaatactgctgtcaatgctacaaaatcatgccgggtcctgtgcatggccgtctgaggaggttcttctggtagaagtttaaaaggtctctgggcgacgggtgtaacttgccaatttcccctacatccgaacatggcagatgaacagaaggaactcgcaaccaacgtagccgaccatggtcttactggccaacttccctcatcaaacgaaaccacggagggactcggagtcacgcaagactgctcttgctacatcacgctccacaatgggaccgaccatgagcttgtgctcgtctacgctcaagagaaacacggtgaatggaagacccgccctgcggaaaccgtgagccagaagagcaatatcaagttttggctcaaagacttattccttggtcctggagcagagggtatggtgaagtatcgaatcggaagtaccgagcacaaggtgcagatgaacttcagctgtcctatgtcttctcccaactcggcgtcctggagtcaaggtgaacatgagattccaggcatctggttgccctgtccggaatacaataaatctgatgcgttgcatgccgtgtttgaagtacaacctgggaattaaggcgtcggggcggggagacgtactataccccattgtcgatagcctctggaagtgtcatcataatgactgtttgttttgtcattgaccggcgacttgtcattttgagttcgtttcccttggcctgaggcgcacttaccgggcatcgtcatagagctactgcttaccacaaa

SEQ ID NO: 6 - DNA, 464 bp, Pisolithus tincturius
atggcagatgaacagaaggaactcgcaaccaacgtagccgaccatggtcttactggccaacttccctcatcaaacgaaaccacggagggactcggagtcacgcaagactgctcttgctacatcacgctccacaatgggaccgaccatgagcttgtgctcgtctacgctcaagagaaacacggtgaatggaagacccgccctgcggaaaccgtgagccagaagagcaatatcaagttttggctcaaagacttattccttggtcctggagcagagggtatggtgaagtatcgaatcggaagtaccgagcacaaggtgcagatgaacttcagctgtcctatgtcttctcccaactcggcgtcctggagtcaaggtgaacatgagattccaggcatctggttgccctgtccggaatacaataaatctgatgcgttgcatgccgtgtttgaagtacaacctgggaatta

SEQ ID NO: 7 - protein, 154 aa, Pisolithus tincturius
MADEQKELATNVADHGLTGQLPSSNETTEGLGVTQDCSCYITLHNGTDHELVLVYAQEKHGEWKTRPAETVSQKSNIKFWLKDLFLGPGAEGMVKYRIGSTEHKVQMNFSCPMSSPNSASWSQGEHEIPGIWLPCPEYNKSDALHAVFEVQPGN

SEQ ID NO: 8 - protein, 121 aa, Artificial Sequence
  Mutated protein from Mattirolomyces terfezioides
MPDLSSFITIKHNSHHVFTRTAIYSKYAAVQWSQEPHLSISPGKWDLFILKDILSIRGTSGYVQYRVGAAQGWVRVTFSSLVGADEVAEWSSGDLPDGFVWHQQVTTGSRPLQATFEATKQ

SEQ ID NO: 9 - protein, 121 aa, Artificial Sequence
  Mutated protein from Mattirolomyces terfezioides
MPDLSSFITIKNNTDHVFTRTAIYSKYAAVQWSPQPQLSISHGKWDLFILKDILSIRGTSGYVQYRVGHGPDWVRVTFSSLVGADEVAEWSSGDLPDGFVWHEHVPMGSRPLQATFEATKQ

SEQ ID NO: 10 - protein, 121 aa, Artificial Sequence
  Mutated protein from Mattirolomyces terfezioides
MPDLSSFITIKNKPNHVFTRTAIYSKYAAVQWSSESQLSIPSGEWDLFILKDILSIRGTSGYVQYRVGVGSCWVRVTFSSLVGADEVAEWSSGDLPDGFVLQKSVQTGSRPLQATFEATKQ

SEQ ID NO: 11 - protein, 121 aa, Artificial Sequence
  Mutated protein from Mattirolomyces terfezioides
MPDLSSFITIKNHTNRVFTRTAIYSKYAAVQWTPESLMSISPGTWDLFILKDILSIRGTSGYVQYRVGDCPGWVRVTFSSLVGADEVAEWSSGDLPDGFVLQKPVQMGTRPLQATFEATKQ

SEQ ID NO: 12 - protein, 121 aa, Artificial Sequence
  Mutated protein from Mattirolomyces terfezioides
MPDLSSFITIKDNSNQVFTRTAIYSKYAAVQWCPELPRSISLGKWDLFILKDILSIRGTSGYVQYRVGDALAWVRVTFSSLVGADEVAEWSSGDLPDGFVLQKLVRNGSRPLQATFEATKQ

SEQ ID NO: 13 - protein, 121 aa, Artificial Sequence
  Mutated protein from Mattirolomyces terezoides
MPDLSSFITIKHNAHHVFTRTAIYSKYAAVQWSQEQQLSIAPGTWDLFILKDILSIRGTSGYVQYRVRDGPGWVRVTFSSLVGADEVAEWSSGDLPDGFVLQKQVRKRARPLQATFEATKQ

SEQ ID NO: 14 - protein, 121 aa, Artificial Sequence
  Mutated protein from Mattirolomyces terfezioides
MPDLSSFITIKNHSNNVFTRTAIYSKYAAVQWPRGPLLSISPRQWDLFILKDILSIRGTSGYVQYRVGDGRGWVRVTFSSLVGADEVAEWSSGDLPDGFVLQKRVGNGSRPLQATFEATKQ

SEQ ID NO: 15 - protein, 121 aa, Artificial Sequence
  Mutated protein from Mattirolomyces terfezioides
MPDLSSFITIKNNSNHVFTRTAIYSKYAAVQWSHQPRPSIWPDMWDLFILKDILSIRGTSGYVQYRVGDDPGWVRVTFSSLVGADEVAEWSSGDLPDGFVLRMPDPTGSRPLQATFEATKQ

SEQ ID NO: 16 - protein, 121 aa, Artificial Sequence
  Mutated protein from Mattirolomyces terfezioides
MPDLSSFITIKDDPNQVFTRTAIYSKYAAVQWSPEHQFSISPGKWDLFILKDILSIRGTSGYVQYRVCDCPGWVRVTFSSLVGADEVAEWSSGDLPDGFVFQTPVTTGPRPLQATFEATKQ

SEQ ID NO: 17 - protein, 121 aa, Artificial Sequence
  Mutated protein from Mattirolomyces terfezioides
MPDLSSFITIKNKTNHVFTRTAIYSKYAAVQWTQQPQISITQGKWDLFILKDILSIRGTSGYVQYRVGDDPGWVRVTFSSLVGADEVAEWSSGDLPDGFVLRKPLRMGSRPLQATFEATKQ

SEQ ID NO: 18 - DNA, 58 bp, Artificial Sequence
  Synthetic Adapter Sequence
aatgatacggcgaccaccgagatctacactctttccctacacgacgctcttccgatct

SEQ ID NO: 19 - DNA, 58 bp, Artificial Sequence
  Synthetic Adapter Sequence
  misc_feature (34)..(34): insertion of i7 barcode
gatcggaagagcacacgtctgaactccagtcacnatctcgtatgccgtcttctgcttg

SEQ ID NO: 20 - DNA, 384 bp, Artificial Sequence
  Modified coding sequence for E. coli expression for protein from Mattirolomyces terfezioides with His-Tag
  CDS (1)..(384)
atgccggatttgagctcgttcattactattaagaataactctaaccatgtttttacgcgtaccgcaatctattccaaatatgccgcagtccagtggagcccggaaccgcagctgagcattagcccaggtaaatgggacctgttcatcctgaaagacatcctgagcatccgcggtacgtccggctacgtgcagtaccgtgtcggcgacggtccgggctgggtgcgtgttacctttagcagcctggtgggtgcggacgaagttgctgagtggagcagcggtgatctgccggatggctttgttctgcaaaagcctgtccgcaccggtagccgtccgctgcaagcgacgttcgaggcgaccaagcaacatcaccatcaccaccactaa

SEQ ID NO: 21 - protein, 127 aa, Artificial Sequence
  Synthetic Construct
MPDLSSFITIKNNSNHVFTRTAIYSKYAAVQWSPEPQLSISPGKWDLFILKDILSIRGTSGYVQYRVGDGPGWVRVTFSSLVGADEVAEWSSGDLPDGFVLQKPVRTGSRPLQATFEATKQHHHHHH

SEQ ID NO: 22 - DNA, 366 bp, Artificial Sequence
  Modified coding sequence for Saccharomyces cerevisiae expression for protein from Mattirolomyces terfezioides with His-Tag
atgcctgatttatcaagttttatcaccattaaaaataactctaaccatgtttttactagaacagccatctactcaaagtacgcagccgtccaatggtccccagaacctcagttgtctatatctccaggtaaatgggatcttttcatcttaaaagatattctaagtattagaggcacttctggttacgtacagtatcgtgttggtgatggacctggttgggttagagtaacattcagctcattggttggggctgacgaagtggctgagtggtcctcaggtgacctcccagatggcttcgtgctgcaaaagccagtcagaactggatctagaccattgcaagcgacattcgaagcaacaaagcaatga

SEQ ID NO: 23 - DNA, 384 bp, Artificial Sequence
  Coding Sequence for modfied protein from Mattirolomyces terfezioides including His-Tag
atgccggaattgagctcgttcattactattaagaataactctaaccatgtttttacgcgtaccgcaatctattccaaatatgccgcagtccagtggagcccggaaccgcagctgagcattagcccaggtaaatgggacctgttcatcctgaaagacatcctgagcatccgcggtacgtccggctacgtgcagtaccgtgtcggcgacggtccgggctgggtgcgtgttacctttagcagcctggtgggtgcggacgaagttgctgagtggagcagcggtgatctgccggatggctttgttctgcaaaagcctgtccgcaccggtagccgtccgctgcaagcgacgttcgaggcgaccaagcaacatcaccaccaccaccactaa

SEQ ID NO: 24 - protein, 127 aa, Artificial Sequence
  Modified protein from Mattirolomyces terfezioides with optional His-Tag
  misc_feature (122)..(127): Absent or Histidine
MPELSSFITIKNNSNHVFTRTAIYSKYAAVQWSPEPQLSISPGKWDLFILKDILSIRGTSGYVQYRVGDGPGWVRVTFSSLVGADEVAEWSSGDLPDGFVLQKPVRTGSRPLQATFEATKQXXXXXX

SEQ ID NO: 25 - DNA, 384 bp, Artificial Sequence
  Coding Sequence of modified protein from Mattirolomyces terfezioides with His-Tag
atgccggatttgagctcgttcattactattagaaataactctaaccatgtttttacgcgtaccgcaatctattccaaatatgccgcagtccagtggagcccggaaccgcagctgagcattagcccaggtaaatgggacctgttcatcctgaaagacatcctgagcatccgcggtacgtccggctacgtgcagtaccgtgtcggcgacggtccgggctgggtgcgtgttacctttagcagcctggtgggtgcggacgaagttgctgagtggagcagcggtgatctgccggatggctttgttctgcaaaagcctgtccgcaccggtagccgtccgctgcaagcgacgttcgaggcgaccaagcaacatcaccaccaccaccactaa

SEQ ID NO: 26 - protein, 127 aa, Artificial Sequence
  Modified protein from Mattirolomyces terfezioides with optional His-Tag
  misc_feature (122)..(127): Absnet or Histidine
MPDLSSFITIRNNSNHVFTRTAIYSKYAAVQWSPEPQLSISPGKWDLFILKDILSIRGTSGYVQYRVGDGPGWVRVTFSSLVGADEVAEWSSGDLPDGFVLQKPVRTGSRPLQATFEATKQXXXXXX

SEQ ID NO: 27 - DNA, 384 bp, Artificial Sequence
  Coding Sequence of modified protein from Mattirolomyces terfezioides with His-Tag
atgccggatttgagctcgttcattactattaagaataactctaaccatgtttttacgaaaaccgcaatctattccaaatatgccgcagtccagtggagcccggaaccgcagctgagcattagcccaggtaaatgggacctgttcatcctgaaagacatcctgagcatccgcggtacgtccggctacgtgcagtaccgtgtcggcgacggtccgggctgggtgcgtgttacctttagcagcctggtgggtgcggacgaagttgctgagtggagcagcggtgatctgccggatggctttgttctgcaaaagcctgtccgcaccggtagccgtccgctgcaagcgacgttcgaggcgaccaagcaacatcaccaccaccaccactaa

SEQ ID NO: 28 - protein, 127 aa, Artificial Sequence
  Modified protein from Mattirolomyces terfezioides with optional His-Tag
  misc_feature (122)..(127): Absent or Histidine
MPDLSSFITIKNNSNHVFTKTAIYSKYAAVQWSPEPQLSISPGKWDLFILKDILSIRGTSGYVQYRVGDGPGWVRVTFSSLVGADEVAEWSSGDLPDGFVLQKPVRTGSRPLQATFEATKQXXXXXX

SEQ ID NO: 29 - DNA, 384 bp, Artificial Sequence
  Coding Sequence of modified protein from Mattirolomyces terfezioides with His-Tag
atgccggatttgagctcgttcattactattaagaataactctaaccatgtttttacgcgtaccgcaatctattcccgctatgccgcagtccagtggagcccggaaccgcagctgagcattagcccaggtaaatgggacctgttcatcctgaaagacatcctgagcatccgcggtacgtccggctacgtgcagtaccgtgtcggcgacggtccgggctgggtgcgtgttacctttagcagcctggtgggtgcggacgaagttgctgagtggagcagcggtgatctgccggatggctttgttctgcaaaagcctgtccgcaccggtagccgtccgctgcaagcgacgttcgaggcgaccaagcaacatcaccaccaccaccactaa

SEQ ID NO: 30 - protein, 127 aa, Artificial Sequence
  Modified protein from Mattirolomyces terfezioides with optional His-Tag
  misc_feature (122)..(127): Absent or Histidine
MPDLSSFITIKNNSNHVFTRTAIYSRYAAVQWSPEPQLSISPGKWDLFILKDILSIRGTSGYVQYRVGDGPGWVRVTFSSLVGADEVAEWSSGDLPDGFVLQKPVRTGSRPLQATFEATKQXXXXXX

SEQ ID NO: 31 - DNA, 384 bp, Artificial Sequence
  Coding Sequence of modified protein from Mattirolomyces terfezioides with His-Tag
atgccggatttgagctcgttcattactattaagaataactctaaccatgtttttacgcgtaccgcaatctattccaaatatgccgcagtccagtggagcccggatccgcagctgagcattagcccaggtaaatgggacctgttcatcctgaaagacatcctgagcatccgcggtacgtccggctacgtgcagtaccgtgtcggcgacggtccgggctgggtgcgtgttacctttagcagcctggtgggtgcggacgaagttgctgagtggagcagcggtgatctgccggatggctttgttctgcaaaagcctgtccgcaccggtagccgtccgctgcaagcgacgttcgaggcgaccaagcaacatcaccaccaccaccactaa

SEQ ID NO: 32 - protein, 127 aa, Artificial Sequence
  Modified protein from Mattirolomyces terfezioides with optional His-Tag
  misc_feature (122)..(127): Absent or Histidine
MPDLSSFITIKNNSNHVFTRTAIYSKYAAVQWSPDPQLSISPGKWDLFILKDILSIRGTSGYVQYRVGDGPGWVRVTFSSLVGADEVAEWSSGDLPDGFVLQKPVRTGSRPLQATFEATKQXXXXXX

SEQ ID NO: 33 - DNA, 384 bp, Artificial Sequence
  Coding Sequence of modified protein from Mattirolomyces terfezioides with His-Tag
atgccggatttgagctcgttcattactattaagaataactctaaccatgtttttacgcgtaccgcaatctattccaaatatgccgcagtccagtggagcccggaaccgcagctgagcattagcccaggtcgctgggacctgttcatcctgaaagacatcctgagcatccgcggtacgtccggctacgtgcagtaccgtgtcggcgacggtccgggctgggtgcgtgttacctttagcagcctggtgggtgcggacgaagttgctgagtggagcagcggtgatctgccggatggctttgttctgcaaaagcctgtccgcaccggtagccgtccgctgcaagcgacgttcgaggcgaccaagcaacatcaccaccaccaccactaa

SEQ ID NO: 34 - protein, 127 aa, Artificial Sequence
  Modified protein from Mattirolomyces terfezioides with optional His-Tag
  misc_feature (122)..(127): Absent or Histidine
MPDLSSFITIKNNSNHVFTRTAIYSKYAAVQWSPEPQLSISPGRWDLFILKDILSIRGTSGYVQYRVGDGPGWVRVTFSSLVGADEVAEWSSGDLPDGFVLQKPVRTGSRPLQATFEATKQXXXXXX

SEQ ID NO: 35 - DNA, 384 bp, Artificial Sequence
  Coding Sequence of modified protein from Mattirolomyces terfezioides with His-Tag
atgccggatttgagctcgttcattactattaagaataactctaaccatgtttttacgcgtaccgcaatctattccaaatatgccgcagtccagtggagcccggaaccgcagctgagcattagcccaggtaaatgggaactgttcatcctgaaagacatcctgagcatccgcggtacgtccggctacgtgcagtaccgtgtcggcgacggtccgggctgggtgcgtgttacctttagcagcctggtgggtgcggacgaagttgctgagtggagcagcggtgatctgccggatggctttgttctgcaaaagcctgtccgcaccggtagccgtccgctgcaagcgacgttcgaggcgaccaagcaacatcaccaccaccaccactaa

SEQ ID NO: 36 - protein, 127 aa, Artificial Sequence
  Modified protein from Mattirolomyces terfezioides with optional His-Tag
  misc_feature (122)..(127): Absent or Histidine
MPDLSSFITIKNNSNHVFTRTAIYSKYAAVQWSPEPQLSISPGKWELFILKDILSIRGTSGYVQYRVGDGPGWVRVTFSSLVGADEVAEWSSGDLPDGFVLQKPVRTGSRPLQATFEATKQXXXXXX

SEQ ID NO: 37 - DNA, 384 bp, Artificial Sequence
  Coding Sequence of modified protein from Mattirolomyces terfezioides with His-Tag
atgccggatttgagctcgttcattactattaagaataactctaaccatgtttttacgcgtaccgcaatctattccaaatatgccgcagtccagtggagcccggaaccgcagctgagcattagcccaggtaaatgggacctgttcatcctgcgcgacatcctgagcatccgcggtacgtccggctacgtgcagtaccgtgtcggcgacggtccgggctgggtgcgtgttacctttagcagcctggtgggtgcggacgaagttgctgagtggagcagcggtgatctgccggatggctttgttctgcaaaagcctgtccgcaccggtagccgtccgctgcaagcgacgttcgaggcgaccaagcaacatcaccaccaccaccactaa

SEQ ID NO: 38 - protein, 127 aa, Artificial Sequence
  Modified protein from Mattirolomyces terfezioides with optional His-Tag
  misc_feature (122)..(127): Absent or Histidine
MPDLSSFITIKNNSNHVFTRTAIYSKYAAVQWSPEPQLSISPGKWDLFILRDILSIRGTSGYVQYRVGDGPGWVRVTFSSLVGADEVAEWSSGDLPDGFVLQKPVRTGSRPLQATFEATKQXXXXXX

SEQ ID NO: 39 - DNA, 384 bp, Artificial Sequence
  Coding Sequence of modified protein from Mattirolomyces terfezioides with His-Tag
atgccggatttgagctcgttcattactattaagaataactctaaccatgtttttacgcgtaccgcaatctattccaaatatgccgcagtccagtggagcccggaaccgcagctgagcattagcccaggtaaatgggacctgttcatcctgaaagaaatcctgagcatccgcggtacgtccggctacgtgcagtaccgtgtcggcgacggtccgggctgggtgcgtgttacctttagcagcctggtgggtgcggacgaagttgctgagtggagcagcggtgatctgccggatggctttgttctgcaaaagcctgtccgcaccggtagccgtccgctgcaagcgacgttcgaggcgaccaagcaacatcaccaccaccaccactaa

SEQ ID NO: 40 - protein, 127 aa, Artificial Sequence
  Modified protein from Mattirolomyces terfezioides with optional His-Tag
  misc_feature (122)..(127): Absent or Histidine
MPDLSSFITIKNNSNHVFTRTAIYSKYAAVQWSPEPQLSISPGKWDLFILKEILSIRGTSGYVQYRVGDGPGWVRVTFSSLVGADEVAEWSSGDLPDGFVLQKPVRTGSRPLQATFEATKQXXXXXX

SEQ ID NO: 41 - DNA, 384 bp, Artificial Sequence
  Coding Sequence of modified protein from Mattirolomyces terfezioides with His-Tag
atgccggatttgagctcgttcattactattaagaataactctaaccatgtttttacgcgtaccgcaatctattccaaatatgccgcagtccagtggagcccggaaccgcagctgagcattagcccaggtaaatgggacctgttcatcctgaaagacatcctgagcatcaaaggtacgtccggctacgtgcagtaccgtgtcggcgacggtccgggctgggtgcgtgttacctttagcagcctggtgggtgcggacgaagttgctgagtggagcagcggtgatctgccggatggctttgttctgcaaaagcctgtccgcaccggtagccgtccgctgcaagcgacgttcgaggcgaccaagcaacatcaccaccaccaccactaa

SEQ ID NO: 42 - protein, 127 aa, Artificial Sequence
  Modified protein from Mattirolomyces terfezioides with optional His-Tag
  misc_feature (122)..(127): Absent or Histidine
MPDLSSFITIKNNSNHVFTRTAIYSKYAAVQWSPEPQLSISPGKWDLFILKDILSIKGTSGYVQYRVGDGPGWVRVTFSSLVGADEVAEWSSGDLPDGFVLQKPVRTGSRPLQATFEATKQXXXXXX

SEQ ID NO: 43 - DNA, 384 bp, Artificial Sequence
  Coding Sequence of modified protein from Mattirolomyces terfezioides with His-Tag
atgccggatttgagctcgttcattactattaagaataactctaaccatgtttttacgcgtaccgcaatctattccaaatatgccgcagtccagtggagcccggaaccgcagctgagcattagcccaggtaaatgggacctgttcatcctgaaagacatcctgagcatccgcggtacgtccggctacgtgcagtacaaagtcggcgacggtccgggctgggtgcgtgttacctttagcagcctggtgggtgcggacgaagttgctgagtggagcagcggtgatctgccggatggctttgttctgcaaaagcctgtccgcaccggtagccgtccgctgcaagcgacgttcgaggcgaccaagcaacatcaccaccaccaccactaa

SEQ ID NO: 44 - protein, 127 aa, Artificial Sequence
  Modified protein from Mattirolomyces terfezioides with optional His-Tag
  misc_feature (122)..(127): Absent or Histidine
MPDLSSFITIKNNSNHVFTRTAIYSKYAAVQWSPEPQLSISPGKWDLFILKDILSIRGTSGYVQYKVGDGPGWVRVTFSSLVGADEVAEWSSGDLPDGFVLQKPVRTGSRPLQATFEATKQXXXXXX

SEQ ID NO: 45 - DNA, 384 bp, Artificial Sequence
  Coding Sequence of modified protein from Mattirolomyces terfezioides with His-Tag
atgccggatttgagctcgttcattactattaagaataactctaaccatgtttttacgcgtaccgcaatctattccaaatatgccgcagtccagtggagcccggaaccgcagctgagcattagcccaggtaaatgggacctgttcatcctgaaagacatcctgagcatccgcggtacgtccggctacgtgcagtaccgtgtcggcgagggtccgggctgggtgcgtgttacctttagcagcctggtgggtgcggacgaagttgctgagtggagcagcggtgatctgccggatggctttgttctgcaaaagcctgtccgcaccggtagccgtccgctgcaagcgacgttcgaggcgaccaagcaacatcaccaccaccaccactaa

SEQ ID NO: 46 - protein, 127 aa, Artificial Sequence
  Modified protein from Mattirolomyces terfezioides with optional His-Tag
  misc_feature (122)..(127): Absent or Histidine
MPDLSSFITIKNNSNHVFTRTAIYSKYAAVQWSPEPQLSISPGKWDLFILKDILSIRGTSGYVQYRVGEGPGWVRVTFSSLVGADEVAEWSSGDLPDGFVLQKPVRTGSRPLQATFEATKQXXXXXX

SEQ ID NO: 47 - DNA, 384 bp, Artificial Sequence
  Coding Sequence of modified protein from Mattirolomyces terfezioides with His-Tag
atgccggatttgagctcgttcattactattaagaataactctaaccatgtttttacgcgtaccgcaatctattccaaatatgccgcagtccagtggagcccggaaccgcagctgagcattagcccaggtaaatgggacctgttcatcctgaaagacatcctgagcatccgcggtacgtccggctacgtgcagtaccgtgtcggcgacggtccgggctgggtgaaagttacctttagcagcctggtgggtgcggacgaagttgctgagtggagcagcggtgatctgccggatggctttgttctgcaaaagcctgtccgcaccggtagccgtccgctgcaagcgacgttcgaggcgaccaagcaacatcaccaccaccaccactaa

SEQ ID NO: 48 - protein, 127 aa, Artificial Sequence
  Modified protein from Mattirolomyces terfezioides with optional His-Tag
  misc_feature (122)..(127): Absent or Histidine
MPDLSSFITIKNNSNHVFTRTAIYSKYAAVQWSPEPQLSISPGKWDLFILKDILSIRGTSGYVQYRVGDGPGWVKVTFSSLVGADEVAEWSSGDLPDGFVLQKPVRTGSRPLQATFEATKQXXXXXX

SEQ ID NO: 49 - DNA, 384 bp, Artificial Sequence
  Coding Sequence of modified protein from Mattirolomyces terfezioides with His-Tag
atgccggatttgagctcgttcattactattaagaataactctaaccatgtttttacgcgtaccgcaatctattccaaatatgccgcagtccagtggagcccggaaccgcagctgagcattagcccaggtaaatgggacctgttcatcctgaaagacatcctgagcatccgcggtacgtccggctacgtgcagtaccgtgtcggcgacggtccgggctgggtgcgtgttacctttagcagcctggtgggtgcggaagaagttgctgagtggagcagcggtgatctgccggatggctttgttctgcaaaagcctgtccgcaccggtagccgtccgctgcaagcgacgttcgaggcgaccaagcaacatcaccaccaccaccactaa

SEQ ID NO: 50 - protein, 127 aa, Artificial Sequence
  Modified protein from Mattirolomyces terfezioides with optional His-Tag
  misc_feature (122)..(127): Absent or Histidine
MPDLSSFITIKNNSNHVFTRTAIYSKYAAVQWSPEPQLSISPGKWDLFILKDILSIRGTSGYVQYRVGDGPGWVRVTFSSLVGAEEVAEWSSGDLPDGFVLQKPVRTGSRPLQATFEATKQXXXXXX

SEQ ID NO: 51 - DNA, 384 bp, Artificial Seguence
  Coding Sequence of modified protein from Mattirolomyces terfezioides with His-Tag
atgccggatttgagctcgttcattactattaagaataactctaaccatgtttttacgcgtaccgcaatctattccaaatatgccgcagtccagtggagcccggaaccgcagctgagcattagcccaggtaaatgggacctgttcatcctgaaagacatcctgagcatccgcggtacgtccggctacgtgcagtaccgtgtcggcgacggtccgggctgggtgcgtgttacctttagcagcctggtgggtgcggacgatgttgctgagtggagcagcggtgatctgccggatggctttgttctgcaaaagcctgtccgcaccggtagccgtccgctgcaagcgacgttcgaggcgaccaagcaacatcaccaccaccaccactaa

SEQ ID NO: 52 - protein, 127 aa, Artificial Sequence
  Modified protein from Mattirolomyces terfezioides with optional His-Tag
  misc_feature (122)..(127): Absent or Histidine
MPDLSSFITIKNNSNHVFTRTAIYSKYAAVQWSPEPQLSISPGKWDLFILKDILSIRGTSGYVQYRVGDGPGWVRVTFSSLVGADDVAEWSSGDLPDGFVLQKPVRTGSRPLQATFEATKQXXXXXX

SEQ ID NO: 53 - DNA, 384 bp, Artificial Sequence
  Coding Sequence of modified protein from Mattirolomyces terfezioides with His-Tag
atgccggatttgagctcgttcattactattaagaataactctaaccatgtttttacgcgtaccgcaatctattccaaatatgccgcagtccagtggagcccggaaccgcagctgagcattagcccaggtaaatgggacctgttcatcctgaaagacatcctgagcatccgcggtacgtccggctacgtgcagtaccgtgtcggcgacggtccgggctgggtgcgtgttacctttagcagcctggtgggtgcggacgaagttgctgattggagcagcggtgatctgccggatggctttgttctgcaaaagcctgtccgcaccggtagccgtccgctgcaagcgacgttcgaggcgaccaagcaacatcaccaccaccaccactaa

SEQ ID NO: 54 - protein, 127 aa, Artificial Sequence
  Modified protein from Mattirolomyces terfezioides with optional His-Tag
  misc_feature (122)..(127): Absent or Histidine
MPDLSSFITIKNNSNHVFTRTAIYSKYAAVQWSPEPQLSISPGKWDLFILKDILSIRGTSGYVQYRVGDGPGWVRVTFSSLVGADEVADWSSGDLPDGFVLQKPVRTGSRPLQATFEATKQXXXXXX

SEQ ID NO: 55 - DNA, 384 bp, Artificial Sequence
  Coding Sequence of modified protein from Mattirolomyces terfezioides with His-Tag
atgccggatttgagctcgttcattactattaagaataactctaaccatgtttttacgcgtaccgcaatctattccaaatatgccgcagtccagtggagcccggaaccgcagctgagcattagcccaggtaaatgggacctgttcatcctgaaagacatcctgagcatccgcggtacgtccggctacgtgcagtaccgtgtcggcgacggtccgggctgggtgcgtgttacctttagcagcctggtgggtgcggacgaagttgctgagtggagcagcggtgagctgccggatggctttgttctgcaaaagcctgtccgcaccggtagccgtccgctgcaagcgacgttcgaggcgaccaagcaacatcaccaccaccaccactaa

SEQ ID NO: 56 - protein, 127 aa, Artificial Sequence
  Modified protein from Mattirolomyces terfezioides with optional His-Tag
  misc_feature (122)..(127): Absent or Histidine
MPDLSSFITIKNNSNHVFTRTAIYSKYAAVQWSPEPQLSISPGKWDLFILKDILSIRGTSGYVQYRVGDGPGWVRVTFSSLVGADEVAEWSSGELPDGFVLQKPVRTGSRPLQATFEATKQXXXXXX

SEQ ID NO: 57 - DNA, 384 bp, Artificial Sequence
  Coding Sequence of modified protein from Mattirolomyces terfezioides with His-Tag
atgccggatttgagctcgttcattactattaagaataactctaaccatgtttttacgcgtaccgcaatctattccaaatatgccgcagtccagtggagcccggaaccgcagctgagcattagcccaggtaaatgggacctgttcatcctgaaagacatcctgagcatccgcggtacgtccggctacgtgcagtaccgtgtcggcgacggtccgggctgggtgcgtgttacctttagcagcctggtgggtgcggacgaagttgctgagtggagcagcggtgatctgccggaaggctttgttctgcaaaagcctgtccgcaccggtagccgtccgctgcaagcgacgttcgaggcgaccaagcaacatcaccaccaccaccactaa

SEQ ID NO: 58 - protein, 127 aa, Artificial Sequence
  Modified protein from Mattirolomyces terfezioides with optional His-Tag
  misc_feature (122)..(127): Absent or Histidine
MPDLSSFITIKNNSNHVFTRTAIYSKYAAVQWSPEPQLSISPGKWDLFILKDILSIRGTSGYVQYRVGDGPGWVRVTFSSLVGADEVAEWSSGDLPEGFVLQKPVRTGSRPLQATFEATKQXXXXXX

SEQ ID NO: 59 - DNA, 384 bp, Artificial Sequence
  Coding Sequence of modified protein from Mattirolomyces terfezioides with His-Tag
atgccggatttgagctcgttcattactattaagaataactctaaccatgtttttacgcgtaccgcaatctattccaaatatgccgcagtccagtggagcccggaaccgcagctgagcattagcccaggtaaatgggacctgttcatcctgaaagacatcctgagcatccgcggtacgtccggctacgtgcagtaccgtgtcggcgacggtccgggctgggtgcgtgttacctttagcagcctggtgggtgcggacgaagttgctgagtggagcagcggtgatctgccggatggctttgttctgcaacgccctgtccgcaccggtagccgtccgctgcaagcgacgttcgaggcgaccaagcaacatcaccaccaccaccactaa

SEQ ID NO: 60 - protein, 127 aa, Artificial Sequence
  Modified protein from Mattirolomyces terfezioides with optional His-Tag
  misc_feature (122)..(127): Absent or Histidine
MPDLSSFITIKNNSNHVFTRTAIYSKYAAVQWSPEPQLSISPGKWDLFILKDILSIRGTSGYVQYRVGDGPGWVRVTFSSLVGADEVAEWSSGDLPDGFVLQRPVRTGSRPLQATFEATKQXXXXXX

SEQ ID NO: 61 - DNA, 384 bp, Artificial Sequence
  Coding Sequence of modified protein from Mattirolomyces terfezioides with His-Tag
atgccggatttgagctcgttcattactattaagaataactctaaccatgtttttacgcgtaccgcaatctattccaaatatgccgcagtccagtggagcccggaaccgcagctgagcattagcccaggtaaatgggacctgttcatcctgaaagacatcctgagcatccgcggtacgtccggctacgtgcagtaccgtgtcggcgacggtccgggctgggtgcgtgttacctttagcagcctggtgggtgcggacgaagttgctgagtggagcagcggtgatctgccggatggctttgttctgcaaaagcctgtcaaaaccggtagccgtccgctgcaagcgacgttcgaggcgaccaagcaacatcaccaccaccaccactaa

SEQ ID NO: 62 - protein, 127 aa, Artificial Sequence
  Modified protein from Mattirolomyces terfezioides with optional His-Tag
  misc_feature (122)..(127): Absnet or Histidine
MPDLSSFITIKNNSNHVFTRTAIYSKYAAVQWSPEPQLSISPGKWDLFILKDILSIRGTSGYVQYRVGDGPGWVRVTFSSLVGADEVAEWSSGDLPDGFVLQKPVKTGSRPLQATFEATKQXXXXXX

SEQ ID NO: 63 - DNA, 384 bp, Artificial Sequence
  Coding Sequence of modified protein from Mattirolomyces terfezioides with His-Tag
atgccggatttgagctcgttcattactattaagaataactctaaccatgtttttacgcgtaccgcaatctattccaaatatgccgcagtccagtggagcccggaaccgcagctgagcattagcccaggtaaatgggacctgttcatcctgaaagacatcctgagcatccgcggtacgtccggctacgtgcagtaccgtgtcggcgacggtccgggctgggtgcgtgttacctttagcagcctggtgggtgcggacgaagttgctgagtggagcagcggtgatctgccggatggctttgttctgcaaaagcctgtccgcaccggtagcaaaccgctgcaagcgacgttcgaggcgaccaagcaacatcaccaccaccaccactaa

SEQ ID NO: 64 - protein, 127 aa, Artificial Sequence
  Modified protein from Mattirolomyces terfezioides with optional His-Tag
  misc_feature (122)..(127): Absent or Histidine
MPDLSSFITIKNNSNHVFTRTAIYSKYAAVQWSPEPQLSISPGKWDLFILKDILSIRGTSGYVQYRVGDGPGWVRVTFSSLVGADEVAEWSSGDLPDGFVLQKPVRTGSKPLQATFEATKQXXXXXX

SEQ ID NO: 65 - DNA, 384 bp, Artificial Sequence
  Coding Sequence of modified protein from Mattirolomyces terfezioides with His-Tag
atgccggatttgagctcgttcattactattaagaataactctaaccatgtttttacgcgtaccgcaatctattccaaatatgccgcagtccagtggagcccggaaccgcagctgagcattagcccaggtaaatgggacctgttcatcctgaaagacatcctgagcatccgcggtacgtccggctacgtgcagtaccgtgtcggcgacggtccgggctgggtgcgtgttacctttagcagcctggtgggtgcggacgaagttgctgagtggagcagcggtgatctgccggatggctttgttctgcaaaagcctgtccgcaccggtagccgtccgctgcaagcgacgttcgatgcgaccaagcaacatcaccaccaccaccactaa

SEQ ID NO: 66 - protein, 127 aa, Artificial Sequence
  Modified protein from Mattirolomyces terfezioides with optional His-Tag
  misc_feature (122)..(127): Absent or Histidine
MPDLSSFITIKNNSNHVFTRTAIYSKYAAVQWSPEPQLSISPGKWDLFILKDILSIRGTSGYVQYRVGDGPGWVRVTFSSLVGADEVAEWSSGDLPDGFVLQKPVRTGSRPLQATFDATKQXXXXXX

SEQ ID NO: 67 - DNA, 384 bp, Artificial Sequence
  Coding Sequence of modified protein from Mattirolomyces terfezioides with His-Tag
atgccggatttgagctcgttcattactattaagaataactctaaccatgtttttacgcgtaccgcaatctattccaaatatgccgcagtccagtggagcccggaaccgcagctgagcattagcccaggtaaatgggacctgttcatcctgaaagacatcctgagcatccgcggtacgtccggctacgtgcagtaccgtgtcggcgacggtccgggctgggtgcgtgttacctttagcagcctggtgggtgcggacgaagttgctgagtggagcagcggtgatctgccggatggctttgttctgcaaaagcctgtccgcaccggtagccgtccgctgcaagcgacgttcgaggcgacccgccaacatcaccaccaccaccactaa

SEQ ID NO: 68 - protein, 127 aa, Artificial Sequence
  Modified protein from Mattirolomyces terfezioides with optional His-Tag
  misc_feature (122)..(127): Absent or Histidine
MPDLSSFITIKNNSNHVFTRTAIYSKYAAVQWSPEPQLSISPGKWDLFILKDILSIRGTSGYVQYRVGDGPGWVRVTFSSLVGADEVAEWSSGDLPDGFVLQKPVRTGSRPLQATFEATRQXXXXXX

SEQ ID NO: 69 - protein, 5 aa, Artificial Sequence
  Amino Acid Linker
  REPEAT (1)..(5): May be repeated n times, where n is any nteger
GGGGS

SEQ ID NO: 70 - protein, 5 aa, Artificial Sequence
  Amino Acid Linker
  REPEAT (1)..(5): May be repeated n times, where n is any integer
EAAAK

SEQ ID NO: 71 - protein, 121 aa, Artificial Sequence
  Consensus Sequence 1
  misc_feature (3)..(3): Xaa is any amino acid
  misc_feature (11)..(16): Xaa is any amino acid
  misc_feature (26)..(26): Xaa is any amino acid
  misc_feature (33)..(34): Xaa is any amino acid
  misc_feature (36)..(38): Xaa is any amino acid
  misc_feature (41)..(43): Xaa is any amino acid
  misc_feature (51)..(51): Xaa is any amino acid
  misc_feature (57)..(57): Xaa is any amino acid
  misc_feature (66)..(66): Xaa is any amino acid
  misc_feature (68)..(72): Xaa is any amino acid
  misc_feature (85)..(86): Xaa is any amino acid
  misc_feature (89)..(89): Xaa is any amino acid
  misc_feature (97)..(97): Xaa can be any naturally occurring amino acid
  misc_feature (101)..(110): Xaa is any amino acid
  misc_feature (117)..(117): Xaa is any amino acid
  misc_feature (120)..(120): Xaa is any amino acid
MPXLSSFITIXXXXXXVFTRTAIYSXYAAVQWXXEXXXSIXXXKWDLFILXDILSIXGTSGYVQYXVXXXXXWVRVTFSSLVGAXXVAXWSSGDLPXGFVXXXXXXXXXXPLQATFXATXQ

SEQ ID NO: 72 - protein, 121 aa, Artificial Sequence
  Consensus sequence 2
  misc_feature (3)..(3): Xaa is any amino acid
  misc_feature (11)..(16): Xaa is any amino acid
  misc_feature (26)..(26): Xaa is any amino acid
  misc_feature (33)..(33): Xaa is any amino acid
  misc_feature (37)..(38): Xaa is any amino acid
  misc_feature (41)..(41): Xaa is any amino acid
  misc_feature (43)..(43): Xaa is any amino acid
  misc_feature (51)..(51): Xaa is any amino acid
  misc_feature (57)..(57): Xaa is any amino acid
  misc_feature (66)..(66): Xaa is any amino acid
  misc_feature (68)..(70): Xaa is any amino acid
  misc_feature (72)..(72): Xaa is any amino acid
  misc_feature (85)..(86): Xaa is any amino acid
  misc_feature (89)..(89): Xaa is any amino acid
  misc_feature (97)..(97): Xaa is any amino acid
  misc_feature (101)..(103): Xaa is any amino acid
  misc_feature (105)..(110): Xaa is any amino acid
  misc_feature (117)..(117): Xaa is any amino acid
  misc_feature (120)..(120): Xaa is any amino acid
MPXLSSFITIXXXXXXVFTRTAIYSXYAAVQWXPEPXXSIXPXKWDLFILXDILSIXGTSGYVQYXVXXXPXWVRVTFSSLVGAXXVAXWSSGDLPXGFVXXXPXXXXXXPLQATFXATXQ

SEQ ID NO: 73 - protein, 121 aa, Artificial Sequence; identical to SEQ ID NO: 72
  Consensus Sequence 3
  misc_feature (3)..(3): Xaa is Asp, Glu, Asn or Gln
  misc_feature (11)..(11): Xaa is Lys, Arg, or His
  misc_feature (12)..(13): Xaa is Asp, Glu, Asn or Gln
  misc_feature (14)..(14): Xaa is Ser, Cys, Thr. or Met
  misc_feature (15)..(15): Xaa is Asp, Glu, Asn or Gln
  misc_feature (16)..(16): Xaa is Val, Gly, Ala, Leu.or Ile
  misc_feature (26)..(26): Xaa is Lys, Arg, or His
  misc_feature (33)..(33): Xaa is Ser, Cys, Thr. or Met
  misc_feature (37)..(37): Xaa is Asp, Glu, Asn or Gln
  misc_feature (38)..(38): Xaa is Val, Gly, Ala, Leu.or Ile
  misc_feature (41)..(41): Xaa is Ser, Cys, Thr. or Met
  misc_feature (43)..(43): Xaa is Val, Gly, Ala, Leu.or Ile
  misc_feature (51)..(51): Xaa is Lys, Arg, or His
  misc_feature (57)..(57): Xaa is Lys, Arg, or His
  misc_feature (66)..(66): Xaa is Lys, Arg, or His
  misc_feature (68)..(68): Xaa is Val, Gly, Ala, Leu.or Ile
  misc_feature (69)..(69): Xaa is Asp, Glu, Asn or Gln
  misc_feature (70)..(70): Xaa is Val, Gly, Ala, Leu.or Ile
  misc_feature (72)..(72): Xaa is Val, Gly, Ala, Leu.or Ile
  misc_feature (85)..(86): Xaa is Asp, Glu, Asn or Gln
  misc_feature (89)..(89): Xaa is Asp, Glu, Asn or Gln
  misc_feature (97)..(97): Xaa is Asp, Glu, Asn or Gln
  misc_feature (101)..(101): Xaa is Val, Gly, Ala, Leu.or Ile
  misc_feature (102)..(102): Xaa is Asp, Glu, Asn or Gln
  misc_feature (103)..(103): Xaa is Lys, Arg, or His
  misc_feature (105)..(105): Xaa is Val, Gly, Ala, Leu.or Ile
  misc_feature (106)..(106): Xaa is Lys, Arg, or His
  misc_feature (107)..(107): Xaa is Ser, Cys, Thr. or Met
  misc_feature (108)..(108): Xaa is Val, Gly, Ala, Leu.or Ile
  misc_feature (108)..(108): Xaa is Val, Gly, Ala, Leu, or Ile
  misc_feature (109)..(109): Xaa is Ser, Cys, Thr. or Met
  misc_feature (110)..(110): Xaa is Lys, Arg, or His
  misc_feature (117)..(117): Xaa is Asp, Glu, Asn or Gln
  misc_feature (120)..(120): Xaa is Lys, Arg, or His

SEQ ID NO: 74 - protein, 121 aa, Artificial Sequence; identical to SEQ ID NO: 72
  Consensus Sequence 4
  misc_feature (3)..(3): Xaa is Asp or Glu
  misc_feature (11)..(11): Xaa is Lys or Arg
  misc_feature (12)..(13): Xaa is Asn or Gln
  misc_feature (14)..(14): Xaa is Ser or Thr
  misc_feature (15)..(15): Xaa is Asn or Gln
  misc_feature (16)..(16): Xaa is Leu, Val, or Ile
  misc_feature (26)..(26): Xaa is Lys or Arg
  misc_feature (33)..(33): Xaa is Ser or Thr
  misc_feature (37)..(37): Xaa is Asn or Gln
  misc_feature (38)..(38): Xaa is Leu, Val, or Ile
  misc_feature (41)..(41): Xaa is Ser or Thr
  misc_feature (43)..(43): Xaa is Gly or Ala
  misc_feature (51)..(51): Xaa is Lys or Arg
  misc_feature (57)..(57): Xaa is Lys or Arg
  misc_feature (66)..(66): Xaa is Lys or Arg
  misc_feature (68)..(68): Xaa is Gly or Ala
  misc_feature (69)..(69): Xaa is Asp or Glu
  misc_feature (70)..(70): Xaa is Gly or Ala
  misc_feature (72)..(72): Xaa is Gly or Ala
  misc_feature (85)..(86): Xaa is Asp or Glu
  misc_feature (89)..(89): Xaa is Asp or Glu
  misc_feature (97)..(97): Xaa is Asp or Glu
  misc_feature (101)..(101): Xaa is Leu, Val, or Ile
  misc_feature (102)..(102): Xaa is Asn or Gln
  misc_feature (103)..(103): Xaa is Lys or Arg
  misc_feature (105)..(105): Xaa is Leu, Val, or Ile
  misc_feature (106)..(106): Xaa is Lys or Arg
  misc_feature (107)..(107): Xaa is Ser or Thr
  misc_feature (108)..(108): Xaa is Gly or Ala
  misc_feature (109)..(109): Xaa is Ser or Thr
  misc_feature (110)..(110): Xaa is Lys or Arg
  misc_feature (117)..(117): Xaa is Asp or Glu
  misc_feature (120)..(120): Xaa is Lys or Arg

SEQ ID NO: 75 - protein, 121 aa, Artificial Sequence
  Consensus Sequence 5
  misc_feature (3)..(3): Xaa is Asp or Glu
  misc_feature (11)..(11): Xaa is Lys or Arg
  misc_feature (26)..(26): Xaa is Lys or Arg
  misc_feature (51)..(51): Xaa is Lys or Arg
  misc_feature (57)..(57): Xaa is Lys or Arg
  misc_feature (66)..(66): Xaa is Lys or Arg
  misc_feature (69)..(69): Xaa is Asp or Glu
  misc_feature (85)..(85): Xaa is Asp or Glu
  misc_feature (86)..(86): Xaa is Asp or Glu
  misc_feature (89)..(89): Xaa is Asp or Glu
  misc_feature (97)..(97): Xaa is Asp or Glu
  misc_feature (103)..(103): Xaa is Lys or Arg
  misc_feature (106)..(106): Xaa is Lys or Arg
  misc_feature (110)..(110): Xaa is Lys or Arg
  misc_feature (117)..(117): Xaa is Asp or Glu
  misc_feature (120)..(120): Xaa is Lys or Arg
MPXLSSFITIXNNSNHVFTRTAIYSXYAAVQWSPEPQLSISPGKWDLFILXDILSIXGTSGYVQYXVGXGPGWVRVTFSSLVGAXXVAXWSSGDLPXGFVLQXPVXTGSXPLQATFXATXQ